European Patent Application EP 4 317 437 A1, published February 7, 2024. Title: Recombinant polypeptide with carboxylic acid reducing activity. Applicant: Asahi Kasei Corporation. The sequence listing filed with the application follows.

SEQUENCE LISTING (72 sequences)

SEQ ID NO: 1 - protein, 1178 aa, Mycobacterium abscessus
MTETISTAAVPTTDLEEQVKRRIEQVVSNDPQLAALLPEDSVTEAVNEPDLPLVEVIRRLLEGYGDRPALGQRAFEFVTGDDGATVIALKPEYTTVSYRELWERAEAIAAAWHEQGIRDGDFVAQLGFTSTDFASLDVAGLRLGTVSVPLQTGASLQQRNAILEETRPAVFAASIEYLDAAVDSVLATPSVRLLSVFDYHAEVDSQREALEAVRARLESAGRTIVVEALAEALARGRDLPAAPLPSADPDALRLLIYTSGSTGTPKGAMYPQWLVANLWQKKWLTDDVIPSIGVNFMPMSHLAGRLTLMGTLSGGGTAYYIASSDLSTFFEDIALIRPSEVLFVPRVVEMVFQRFQAELDRSLAPGESNSEIAERIKVRIREQDFGGRVLSAGSGSAPLSPEMTEFMESLLQVPLRDGYGSTEAGGVWRDGVLQRPPVTDYKLVDVPELGYFTTDSPHPRGELRLKSETMFPGYYKRPETTADVFDDEGYYKTGDVVAELGPDHLKYLDRVKNVLKLAQGEFVAVSKLEAAYTGSPLVRQIFVYGNSERSFLLAVVVPTPEVLERYADSPDALKPLIQDSLQQVAKDAELQSYEIPRDFIVETVPFTVESGLLSDARKLLRPKLKDHYGERLEALYAELAESQNERLRQLAREAATRPVLETVTDAAAALLGASSSDLAPDVRFIDLGGDSLSALSYSELLRDIFEVDVPVGVINSVANDLAAIARHIEAQRTGAATQPTFASVHGKDATVITAGELTLDKFLDESLLKAAKDVQPATADVKTVLVTGGNGWLGRWLVLDWLERLAPNGGKVYALIRGADAEAARARLDAVYESGDPKLSAHYRQLAQQSLEVIAGDFGDQDLGLSQEVWQKLAKDVDLIVHSGALVNHVLPYSQLFGPNVAGTAEIIKLAISERLKPVTYLSTVGIADQIPVTEFEEDSDVRVMSAERQINDGYANGYGNSKWAGEVLLREAHDLAGLPVRVFRSDMILAHSDYHGQLNVTDVFTRSIQSLLLTGVAPASFYELDADGNRQRAHYDGVPGDFTAASITAIGGVNVVDGYRSFDVFNPHHDGVSMDTFVDWLIDAGYKIARIDDYDQWLARFELALKGLPEQQRQQSVLPLLKMYEKPQPAIDGSALPTAEFSRAVHEAKVGDSGEIPHVTKELILKYASDIQLLGLV

SEQ ID NO: 2 - DNA, 3534 bp, Mycobacterium abscessus
atgactgaaacgatctccacagcggctgtccccactacggatctcgaagagcaggtgaagcgacgcatcgagcaggtcgtgtccaacgatccgcagctggcggcgcttctcccggaagattcggtcaccgaggcggtcaacgagcccgatctaccgctggtcgaggtgatcaggcgactgctggagggctacggtgaccgcccggcactcggccagcgcgccttcgagttcgtcaccggggacgacggtgcgaccgtgatcgcgctgaagcccgaatacaccaccgtctcctaccgcgagttgtgggaacgtgccgaggctatcgctgccgcgtggcacgagcagggcatccgtgacggcgacttcgtcgctcagttgggtttcaccagcacggacttcgcgtcgctcgacgtcgcgggattgcgtctgggcaccgtctcggtgcccctgcagacgggcgcgtcgctgcagcagcgcaacgcgattctcgaagagacccggcccgcagtctttgccgcgagtatcgaataccttgatgccgccgtcgattcggtgcttgcgaccccctcggtgcgactcctctcggttttcgactatcacgcggaggtcgacagccagcgcgaagcgctggaggctgtgcgggcccggcttgagagtgccggccggacgatcgtcgtcgaggccctggcggaggctctcgcgcgggggcgggacctgcccgccgcgccgctgcccagtgcagatcccgatgccttgcgtctgctcatctacacctccggcagcaccggtacccccaagggcgccatgtatccgcaatggctggtcgccaacttgtggcagaagaagtggctcaccgacgatgtgattccgtccataggcgtgaacttcatgcccatgagccacctggcgggtcgcctcactctcatgggcaccctttccggtggcggaaccgcctactacatcgcttcgagcgatctttcgactttcttcgaggacatcgcgctcatccgcccctccgaagtgctcttcgtgccgcgtgtggtggagatggtgttccagcgttttcaggcagaattggaccggtcccttgccccgggtgagagcaactccgagatcgcggagcgaatcaaggtccgcatccgggaacaggacttcggcgggcgtgtgctcagtgctggctccgggtcggccccgttgtctcctgagatgacggagttcatggagtcgctgctgcaggtgccgttgcgcgacgggtatgggtccaccgaggccggtggtgtgtggcgtgacggagtcctgcagcgtccgcccgtcaccgactacaagctggttgacgttccggaactcggatacttcaccacagattcgccgcatccccgtggcgagctgcggttgaagtcggagacgatgttccccggctactacaagcgcccggagaccactgccgatgtcttcgatgacgaggggtactacaagaccggtgacgtggtcgccgagctcgggccggatcacctcaagtacctcgaccgcgtcaagaacgtcctcaagctcgcgcagggagagtttgtcgcggtgtcaaagctggaggccgcttacaccggcagcccgctggtccggcagatctttgtgtacgggaacagtgaacgctcgttcctgctggctgtcgtggtcccgacacccgaagtccttgagcggtacgcagattcgccagatgcgctcaagcccttgatccaggattcgctgcagcaggtcgccaaggacgcggagctgcaatcctatgagataccgcgcgacttcatcgttgagacggtgccgttcaccgtcgagtccggattgctatcggacgcgcgaaagctgctgcgccccaagctgaaggatcactacggagagaggctggaggcgctgtacgccgaactggcggaaagccagaatgagcggctgcgccagttggccagggaggcagccacgcgcccggtcctggagacggtgaccgatgcggccgccgcgctgctgggcgcatcgtcctcggatctggctcctgatgtgcgattcatcgacctcggtggcgactcactgtcggcgctgtcgtactccgagctgctgcgcgacatctttgaggtggacgttccggtgggcgtcatcaacagcgtcgccaacgaccttgccgcgatcgcccggcacatcgaggcgcagcggaccggcgccgctacgcagccgacctttgcgtcggtccacggcaaggacgcgacggtcatcaccgccggtgaactcaccctcgacaagttcttggacgagtcactgttgaaagcggccaaggacgttcagccggcaacggccgatgtcaagaccgttctagtgaccggcggcaacggctggttgggtcgttggctggtgctcgattggctggagcggttggcacccaatggtggcaaggtctacgccctcattcgtggcgccgatgccgaagcagcccgggcacggttggacgccgtgtacgaatcgggtgatcccaagctgtccgcgcattatcgtcagctggcgcaacagagtctggaagttatcgccggcgatttcggcgaccaggatctcggtctatcccaggaagtttggcagaagctggccaaggacgtggacctgatcgtgcactccggtgccttggtgaaccacgtgctgccgtacagccagttgttcggtccgaatgtggcgggtaccgccgagatcatcaagctggcaatttcggagcggctcaagccggtcacctacctgtcgacggtgggcatcgccgaccagattccggtgacggagttcgaggaagactccgatgttcgtgtgatgtcggccgagcgccagatcaatgacggctacgcgaacggatacggcaactcaaaatgggccggcgaggtgctgttgcgggaggctcatgacctagcggggctgccggtgcgtgtgttccgctccgacatgatcctggcgcacagtgactaccacggacagctcaacgtcaccgacgtgttcacccggagcatccagagtctgctgctcaccggtgttgcaccggccagcttctatgaattggatgccgacggcaatcggcagcgcgctcactatgacggtgtgcccggcgatttcaccgccgcatcgatcaccgccatcggcggtgtgaacgtggtagacggttaccgcagcttcgacgtgttcaacccgcaccatgacggtgtctcgatggataccttcgtcgactggctgatcgacgcaggctacaagatcgcgcggatcgacgattacgaccagtggctcgcccggttcgagctggccctcaagggattgcccgagcagcagcggcaacagtcggtgttgccacttctcaagatgtacgagaagccgcaaccggcgatcgacggaagtgcacttccgaccgcagaattcagtcgcgccgtgcacgaggcgaaggtcggagacagcggtgagataccgcacgtcaccaaggagctgatcctcaagtacgccagcgatattcagctgttgggcctggtg

SEQ ID NO: 3 - protein, 1178 aa, Artificial Sequence
  W283R/ A303M
MTETISTAAVPTTDLEEQVKRRIEQVVSNDPQLAALLPEDSVTEAVNEPDLPLVEVIRRLLEGYGDRPALGQRAFEFVTGDDGATVIALKPEYTTVSYRELWERAEAIAAAWHEQGIRDGDFVAQLGFTSTDFASLDVAGLRLGTVSVPLQTGASLQQRNAILEETRPAVFAASIEYLDAAVDSVLATPSVRLLSVFDYHAEVDSQREALEAVRARLESAGRTIVVEALAEALARGRDLPAAPLPSADPDALRLLIYTSGSTGTPKGAMYPQWLVANLWQKKRLTDDVIPSIGVNFMPMSHLMGRLTLMGTLSGGGTAYYIASSDLSTFFEDIALIRPSEVLFVPRVVEMVFQRFQAELDRSLAPGESNSEIAERIKVRIREQDFGGRVLSAGSGSAPLSPEMTEFMESLLQVPLRDGYGSTEAGGVWRDGVLQRPPVTDYKLVDVPELGYFTTDSPHPRGELRLKSETMFPGYYKRPETTADVFDDEGYYKTGDVVAELGPDHLKYLDRVKNVLKLAQGEFVAVSKLEAAYTGSPLVRQIFVYGNSERSFLLAVVVPTPEVLERYADSPDALKPLIQDSLQQVAKDAELQSYEIPRDFIVETVPFTVESGLLSDARKLLRPKLKDHYGERLEALYAELAESQNERLRQLAREAATRPVLETVTDAAAALLGASSSDLAPDVRFIDLGGDSLSALSYSELLRDIFEVDVPVGVINSVANDLAAIARHIEAQRTGAATQPTFASVHGKDATVITAGELTLDKFLDESLLKAAKDVQPATADVKTVLVTGGNGWLGRWLVLDWLERLAPNGGKVYALIRGADAEAARARLDAVYESGDPKLSAHYRQLAQQSLEVIAGDFGDQDLGLSQEVWQKLAKDVDLIVHSGALVNHVLPYSQLFGPNVAGTAEIIKLAISERLKPVTYLSTVGIADQIPVTEFEEDSDVRVMSAERQINDGYANGYGNSKWAGEVLLREAHDLAGLPVRVFRSDMILAHSDYHGQLNVTDVFTRSIQSLLLTGVAPASFYELDADGNRQRAHYDGVPGDFTAASITAIGGVNVVDGYRSFDVFNPHHDGVSMDTFVDWLIDAGYKIARIDDYDQWLARFELALKGLPEQQRQQSVLPLLKMYEKPQPAIDGSALPTAEFSRAVHEAKVGDSGEIPHVTKELILKYASDIQLLGLV

SEQ ID NO: 4 - protein, 1178 aa, Artificial Sequence
  W283R/ L335F
MTETISTAAVPTTDLEEQVKRRIEQVVSNDPQLAALLPEDSVTEAVNEPDLPLVEVIRRLLEGYGDRPALGQRAFEFVTGDDGATVIALKPEYTTVSYRELWERAEAIAAAWHEQGIRDGDFVAQLGFTSTDFASLDVAGLRLGTVSVPLQTGASLQQRNAILEETRPAVFAASIEYLDAAVDSVLATPSVRLLSVFDYHAEVDSQREALEAVRARLESAGRTIVVEALAEALARGRDLPAAPLPSADPDALRLLIYTSGSTGTPKGAMYPQWLVANLWQKKRLTDDVIPSIGVNFMPMSHLAGRLTLMGTLSGGGTAYYIASSDLSTFFEDIAFIRPSEVLFVPRVVEMVFQRFQAELDRSLAPGESNSEIAERIKVRIREQDFGGRVLSAGSGSAPLSPEMTEFMESLLQVPLRDGYGSTEAGGVWRDGVLQRPPVTDYKLVDVPELGYFTTDSPHPRGELRLKSETMFPGYYKRPETTADVFDDEGYYKTGDVVAELGPDHLKYLDRVKNVLKLAQGEFVAVSKLEAAYTGSPLVRQIFVYGNSERSFLLAVVVPTPEVLERYADSPDALKPLIQDSLQQVAKDAELQSYEIPRDFIVETVPFTVESGLLSDARKLLRPKLKDHYGERLEALYAELAESQNERLRQLAREAATRPVLETVTDAAAALLGASSSDLAPDVRFIDLGGDSLSALSYSELLRDIFEVDVPVGVINSVANDLAAIARHIEAQRTGAATQPTFASVHGKDATVITAGELTLDKFLDESLLKAAKDVQPATADVKTVLVTGGNGWLGRWLVLDWLERLAPNGGKVYALIRGADAEAARARLDAVYESGDPKLSAHYRQLAQQSLEVIAGDFGDQDLGLSQEVWQKLAKDVDLIVHSGALVNHVLPYSQLFGPNVAGTAEIIKLAISERLKPVTYLSTVGIADQIPVTEFEEDSDVRVMSAERQINDGYANGYGNSKWAGEVLLREAHDLAGLPVRVFRSDMILAHSDYHGQLNVTDVFTRSIQSLLLTGVAPASFYELDADGNRQRAHYDGVPGDFTAASITAIGGVNVVDGYRSFDVFNPHHDGVSMDTFVDWLIDAGYKIARIDDYDQWLARFELALKGLPEQQRQQSVLPLLKMYEKPQPAIDGSALPTAEFSRAVHEAKVGDSGEIPHVTKELILKYASDIQLLGLV

SEQ ID NO: 5 - DNA, 154 bp, Artificial Sequence
  promoter
tcaagcccaaaggaagagtgaggcgagtcagtcgcgtaatgcttaggcacaggattgatttgtcgcaatgattgacacgattccgcttgacgctgcgtaaggtttttgtaattttacaggcaaccttttattcactaacaaatagctggtggaa

SEQ ID NO: 6 - DNA, 47 bp, Artificial Sequence
  terminator
aaaaaaaaaaaggtgccgtggaaacacggcacctttttttttcttta

SEQ ID NO: 7 - DNA, 25 bp, Artificial Sequence
  primer 1
atgactgaaacgatctccacagcgg

SEQ ID NO: 8 - DNA, 25 bp, Artificial Sequence
  primer 2
ctacaccaggcccaacagctgaata

SEQ ID NO: 9 - DNA, 25 bp, Artificial Sequence
  primer 3
atgatcgagacaattttgcctgctg

SEQ ID NO: 10 - DNA, 20 bp, Artificial Sequence
  primer 4
tcaggcgtacgcgatcgcgg

SEQ ID NO: 11 - DNA, 20 bp, Artificial Sequence
  primer 5
atgatacgcgagcctccgga

SEQ ID NO: 12 - DNA, 23 bp, Artificial Sequence
  primer 6
ttacgcttcttcgacacttactc

SEQ ID NO: 13 - DNA, 25 bp, Artificial Sequence
  primer 7
cttcttctgccacaagttggcgacc

SEQ ID NO: 14 - DNA, 22 bp, Artificial Sequence
  primer 8
tccgaagtgctcttcgtgccgc

SEQ ID NO: 15 - DNA, 22 bp, Artificial Sequence
  primer 9
atgggcagcagccatcaccatc

SEQ ID NO: 16 - DNA, 26 bp, Artificial Sequence
  primer 10
ggtatatctccttattaaagttaaac

SEQ ID NO: 17 - DNA, 35 bp, Artificial Sequence
  primer 11
tttaataaggagatataccatgatacgcgagcctc

SEQ ID NO: 18 - DNA, 35 bp, Artificial Sequence
  primer 12
ggtgatggctgctgcccatttacgcttcttcgaca

SEQ ID NO: 19 - DNA, 25 bp, Artificial Sequence
  primer 13
agcttgcggccgcataatgcttaag

SEQ ID NO: 20 - DNA, 34 bp, Artificial Sequence
  primer 14
atgtatatctccttcttatacttaactaatatac

SEQ ID NO: 21 - DNA, 35 bp, Artificial Sequence
  primer 15
agaaggagatatacatatgactgaaacgatctcca

SEQ ID NO: 22 - DNA, 33 bp, Artificial Sequence
  primer 16
ggtggcagcagcctagctacaccaggcccaaca

SEQ ID NO: 23 - DNA, 200 bp, Artificial Sequence
  synthetic fragment/ Trp283
  misc_feature (17)..(18): n is a, c, g, t or u
cttgtggcagaagaagnnkctcaccgacgatgtgattccgtccataggcgtgaacttcatgcccatgagccacctggcgggtcgcctcactctcatgggcaccctttccggtggcggaaccgcctactacatcgcttcgagcgatctttcgactttcttcgaggacatcgcgctcatccgcccctccgaagtgctcttcg

SEQ ID NO: 24 - DNA, 200 bp, Artificial Sequence
  synthetic fragment/ Leu 284
  misc_feature (20)..(21): n is a, c, g, t or u
cttgtggcagaagaagtggnnkaccgacgatgtgattccgtccataggcgtgaacttcatgcccatgagccacctggcgggtcgcctcactctcatgggcaccctttccggtggcggaaccgcctactacatcgcttcgagcgatctttcgactttcttcgaggacatcgcgctcatccgcccctccgaagtgctcttcg

SEQ ID NO: 25 - DNA, 200 bp, Artificial Sequence
  synthetic fragment/ Ala 303
  misc_feature (77)..(78): n is a, c, g, t or u
cttgtggcagaagaagtggctcaccgacgatgtgattccgtccataggcgtgaacttcatgcccatgagccacctgnnkggtcgcctcactctcatgggcaccctttccggtggcggaaccgcctactacatcgcttcgagcgatctttcgactttcttcgaggacatcgcgctcatccgcccctccgaagtgctcttcg

SEQ ID NO: 26 - DNA, 200 bp, Artificial Sequence
  synthetic fragment/ Leu 306
  misc_feature (86)..(87): n is a, c, g, t or u
cttgtggcagaagaagtggctcaccgacgatgtgattccgtccataggcgtgaacttcatgcccatgagccacctggcgggtcgcnnkactctcatgggcaccctttccggtggcggaaccgcctactacatcgcttcgagcgatctttcgactttcttcgaggacatcgcgctcatccgcccctccgaagtgctcttcg

SEQ ID NO: 27 - DNA, 200 bp, Artificial Sequence
  synthetic fragment/ Leu 335
  misc_feature (173)..(174): n is a, c, g, t or u
cttgtggcagaagaagtggctcaccgacgatgtgattccgtccataggcgtgaacttcatgcccatgagccacctggcgggtcgcctcactctcatgggcaccctttccggtggcggaaccgcctactacatcgcttcgagcgatctttcgactttcttcgaggacatcgcgnnkatccgcccctccgaagtgctcttcg

SEQ ID NO: 28 - DNA, 36 bp, Artificial Sequence
  primer 17
ttgttgaataaatcgtctgtttgccgagaatacgcg

SEQ ID NO: 29 - DNA, 35 bp, Artificial Sequence
  primer 18
tatcgcatgcagatctgcgctaatgggctccagga

SEQ ID NO: 30 - DNA, 35 bp, Artificial Sequence
  primer 19
ttgttgaataaatcgcgcgccagcgctggctgttt

SEQ ID NO: 31 - DNA, 35 bp, Artificial Sequence
  primer 20
tatcgcatgcagatcccgccaatgccggaagagtt

SEQ ID NO: 32 - DNA, 35 bp, Artificial Sequence
  primer 21
ttgttgaataaatcgcgatcgtgatgccgctgtct

SEQ ID NO: 33 - DNA, 35 bp, Artificial Sequence
  primer 22
tatcgcatgcagatcgacaacgtaggctttgttca

SEQ ID NO: 34 - DNA, 35 bp, Artificial Sequence
  primer 23
ttgttgaataaatcgcgccatctcgacactcttga

SEQ ID NO: 35 - DNA, 35 bp, Artificial Sequence
  primer 24
tatcgcatgcagatcgcgaacatcgatgggttagc

SEQ ID NO: 36 - DNA, 35 bp, Artificial Sequence
  primer 25
ttgttgaataaatcgtggcatttgcccttcctgtt

SEQ ID NO: 37 - DNA, 35 bp, Artificial Sequence
  primer 26
tatcgcatgcagatcgtcctgatcctgcaacggaa

SEQ ID NO: 38 - DNA, 35 bp, Artificial Sequence
  primer 27
ttgttgaataaatcgctcataacggtactgcaaac

SEQ ID NO: 39 - DNA, 35 bp, Artificial Sequence
  primer 28
tatcgcatgcagatctcgcagcaggtaagatgatt

SEQ ID NO: 40 - DNA, 35 bp, Artificial Sequence
  primer 29
ttgttgaataaatcgatattcgtcctaacgaacag

SEQ ID NO: 41 - DNA, 35 bp, Artificial Sequence
  primer 30
tatcgcatgcagatctttttgattttcaagtatgt

SEQ ID NO: 42 - DNA, 35 bp, Artificial Sequence
  primer 31
gatctgcatgcgatatctctagaacgcgtaagctt

SEQ ID NO: 43 - DNA, 29 bp, Artificial Sequence
  primer 32
tctcgagccgatttattcaacaaagccgc

SEQ ID NO: 44 - DNA, 25 bp, Artificial Sequence
  primer 33
actttcgttttcgggcatttcgtcc

SEQ ID NO: 45 - DNA, 24 bp, Artificial Sequence
  primer 34
ccaatatgagggcagagaacgatc

SEQ ID NO: 46 - DNA, 20 bp, Artificial Sequence
  primer 35
atgcgctgatgtgataatgc

SEQ ID NO: 47 - DNA, 19 bp, Artificial Sequence
  primer 36
ccttctccttgttgcttta

SEQ ID NO: 48 - DNA, 20 bp, Artificial Sequence
  primer 37
gaggcctttgctgcgactgc

SEQ ID NO: 49 - DNA, 21 bp, Artificial Sequence
  primer 38
agttcctccttttcggatgat

SEQ ID NO: 50 - DNA, 18 bp, Artificial Sequence
  primer 39
atgccggatgcgacgctt

SEQ ID NO: 51 - DNA, 20 bp, Artificial Sequence
  primer 40
tcattttgcatatagcccct

SEQ ID NO: 52 - DNA, 20 bp, Artificial Sequence
  primer 41
tgacctgggcagtaatggtg

SEQ ID NO: 53 - DNA, 25 bp, Artificial Sequence
  primer 42
caggatctccgttgctttatgagtc

SEQ ID NO: 54 - DNA, 24 bp, Artificial Sequence
  primer 43
cgtggtgttgaaagccgattattg

SEQ ID NO: 55 - DNA, 23 bp, Artificial Sequence
  primer 44
cataaacttccagttctccgccc

SEQ ID NO: 56 - DNA, 20 bp, Artificial Sequence
  primer 45
tcgcacactaacagactgaa

SEQ ID NO: 57 - DNA, 20 bp, Artificial Sequence
  primer 46
tgtgtttactcctgattagc

SEQ ID NO: 58 - DNA, 25 bp, Artificial Sequence
  primer 47
tattctcaatccgtttcagcacgcg

SEQ ID NO: 59 - DNA, 21 bp, Artificial Sequence
  primer 48
ttcgggatcaccaccaggccg

SEQ ID NO: 60 - DNA, 20 bp, Artificial Sequence
  primer 49
cggaaatggacgaacagtgg

SEQ ID NO: 61 - DNA, 22 bp, Artificial Sequence
  primer 50
cgtcatcagcgtttaccagatt

SEQ ID NO: 62 - DNA, 20 bp, Artificial Sequence
  primer 51
gcataaacactgtccgcgtc

SEQ ID NO: 63 - DNA, 24 bp, Artificial Sequence
  primer 52
gaaatcgagaaggcagaagcgaaa

SEQ ID NO: 64 - DNA, 20 bp, Artificial Sequence
  primer 53
ggtgcggtcaccattgttcg

SEQ ID NO: 65 - DNA, 20 bp, Artificial Sequence
  primer 54
catatcgcacgccagcagtg

SEQ ID NO: 66 - DNA, 21 bp, Artificial Sequence
  primer 55
ggtgaggatggagagttcatg

SEQ ID NO: 67 - DNA, 21 bp, Artificial Sequence
  primer 56
cagttcgatttgcgccaccag

SEQ ID NO: 68 - DNA, 20 bp, Artificial Sequence
  primer 57
tccgctagtgtgatttcagg

SEQ ID NO: 69 - DNA, 23 bp, Artificial Sequence
  primer 58
gaaattattatgccgccaggcgt

SEQ ID NO: 70 - DNA, 20 bp, Artificial Sequence
  primer 59
ttatggtctgggcgacatgc

SEQ ID NO: 71 - DNA, 22 bp, Artificial Sequence
  primer 60
gcatcatcctggtcatataccc

SEQ ID NO: 72 - protein, 1188 aa, Segniliparus rugosus
MTESQSYETRQARPAGQSLAERVARLVAIDPQAAAAVPDKAVAERATQQGLRLAQRIEAFLSGYGDRPALAQRAFEITKDPITGRAVATLLPKFETVSYRELLERSHAIASELANHAEAPVKAGEFIATIGFTSTDYTSLDIAGVLLGLTSVPLQTGATTDTLKAIAEETAPAVFGASVEHLDNAVTTALATPSVRRLLVFDYRQGVDEDREAVEAARSRLAEAGSAVLVDTLDEVIARGRALPRVALPPATDAGDDSLSLLIYTSGSTGTPKGAMYPERNVAQFWGGIWHNAFDDGDSAPDVPDIMVNFMPLSHVAGRIGLMGTLSSGGTTYFIAKSDLSTFFEDYSLARPTKLFFVPRICEMIYQHYQSELDRIGAADGSPQAEAIKTELREKLLGGRVLTAGSGSAPMSPELTAFIESVLQVHLVDGYGSTEAGPVWRDRKLVKPPVTEHKLIDVPELGYFSTDSPYPRGELAIKTQTILPGYYKRPETTAEVFDEDGFYLTGDVVAEVAPEEFVYVDRRKNVLKLSQGEFVALSKLEAAYGTSPLVRQISVYGSSQRSYLLAVVVPTPEALAKYGDGEAVKSALGDSLQKIAREEGLQSYEVPRDFIIETDPFTIENGILSDAGKTLRPKVKARYGERLEALYAQLAETQAGELRSIRVGAGERPVIETVQRAAAALLGASAAEVDPEAHFSDLGGDSLSALTYSNFLHEIFQVEVPVSVIVSAANNLRSVAAHIEKERSSGSDRPTFASVHGAGATTIRASDLKLEKFLDAQTLAAAPSLPRPASEVRTVLLTGSNGWLGRFLALAWLERLVPQGGKVVVIVRGKDDKAAKARLDSVFESGDPALLAHYEDLADKGLEVLAGDFSDADLGLRKADWDRLADEVDLIVHSGALVNHVLPYSQLFGPNVVGTAEVAKLALTKRLKPVTYLSTVAVAVGVEPSAFEEDGDIRDVSAVRSIDEGYANGYGNSKWAGEVLLREAYEHAGLPVRVFRSDMILAHRKYTGQLNVPDQFTRLILSLLATGIAPKSFYQLDATGGRQRAHYDGIPVDFTAEAITTLGLAGSDGYHSFDVFNPHHDGVGLDEFVDWLVEAGHPISRVDDYAEWLSRFETSLRGLPEAQRQHSVLPLLHAFAQPAPAIDGSPFQTKNFQSSVQEAKVGAEHDIPHLDKALIVKYAEDIKQLGLL